European Patent Application EP 4 365 286 A1, published May 8, 2024. Title: Esterase Mutant and Use thereof. Applicant: ASYMCHEM LABORATORIES (TIANJIN) CO., LTD. The sequence listing filed with the application follows.

SEQUENCE LISTING (2 sequences)

SEQ ID NO: 1 - protein, 264 aa, Rauvolfia serpentina
MHSAANAKQQKHFVLVHGGCLGAWIWYKLKPLLESAGHKVTAVDLSAAGINPRRLDEIHTFRDYSEPLMEVMASIPPDEKVVLLGHSFGGMSLGLAMETYPEKISVAVFMSAMMPDPNHSLTYPFEKYNEKCPADMMLDSQFSTYGNPENPGMSMILGPQFMALKMFQNCSVEDLELAKMLTRPGSLFFQDLAKAKKFSTERYGSVKRAYIFCNEDKSFPVEFQKWFVESVGADKVKEIKEADHMGMLSQPREVCKCLLDISDS

SEQ ID NO: 2 - DNA, 795 bp, Rauvolfia serpentina
  misc_feature (1)..(795): Nucleic acid sequence optimized for codons in Escherichia coli
atgcacagcgctgcaaacgcaaaacaacagaagcacttcgtcctggtccacggtggttgtctgggtgcttggatctggtacaaactgaaacctctgctggagtctgcaggtcataaagtgactgcagttgatctgagcgcagctggtatcaacccacgtcgtctggatgaaattcacactttccgtgattacagcgagccactgatggaagtgatggctagcatcccgccggatgaaaaagtggttctgctgggtcattctttcggtggtatgtctctgggtctggctatggaaacctacccggagaaaatctctgttgctgtgttcatgtccgccatgatgccggatccgaaccactctctgacctatccgtttgaaaagtacaacgagaagtgcccggccgatatgatgctggactctcaattctctacgtacggcaacccggaaaatccgggcatgtctatgatcctgggcccgcagtttatggcgctgaaaatgtttcagaactgtagcgtagaagacctggaactggccaaaatgctgacccgtcctggctccctgtttttccaggacctggcgaaagcgaaaaagttcagcaccgaacgttatggctccgttaaacgcgcgtatattttctgcaacgaagacaaaagcttcccggttgaattccagaaatggttcgtagagtccgttggcgcggacaaagtaaaagaaatcaaagaagcggaccacatgggcatgctgtcccagccgcgcgaagtttgcaaatgcctgctggacatttccgactcctaa